European Patent Specification EP 4 073 098 B1, published September 27, 2023. Title: ULTRA-LONG ACTING INSULIN-FC FUSION PROTEINS AND METHODS OF USE. Applicant: AKSTON BIOSCIENCES CORPORATION. The sequence listing filed with the application follows.

SEQUENCE LISTING (100 sequences)

SEQ ID NO: 1 - protein, 30 aa, Artificial Sequence
  Human insulin B-chain
FVNQHLCGSHLVEALYLVCGERGFFYTPKT

SEQ ID NO: 2 - protein, 21 aa, Artificial Sequence
  Human insulin A-chain
GIVEQCCTSICSLYQLENYCN

SEQ ID NO: 3 - protein, 86 aa, Artificial Sequence
  Human ProInsulin
FVNQHLCGSHLVEALYLVCGERGFFYTPKTRREAEDLQVGQVELGGGPGAGSLQPLALEGSLQKRGIVEQCCTSICSLYQLENYCN

SEQ ID NO: 4 - protein, 57 aa, Artificial Sequence
  Insulin Polypeptide
FVNQHLCGSDLVEALALVCGERGFFYTDPTGGGPRRGIVEQCCHSICSLYQLENYCN

SEQ ID NO: 5 - protein, 58 aa, Artificial Sequence
  Insulin Polypeptide
  Xaa (10)..(10): Xaa is not D
  Xaa (45)..(45): Xaa is not H
  Xaa (58)..(58): Xaa is absent or N
FVNQHLCGSXLVEALELVCGERGFHYGGGGGGSGGGGGIVEQCCXSTCSLDQLENYCX

SEQ ID NO: 6 - protein, 58 aa, Artificial Sequence
  Insulin Polypeptide
  Xaa (58)..(58): Xaa is absent or N
FVNQHLCGSHLVEALELVCGERGFHYGGGGGGSGGGGGIVEQCCTSTCSLDQLENYCX

SEQ ID NO: 7 - protein, 57 aa, Artificial Sequence
  Insulin Polypeptide
FVNQHLCGSHLVEALELVCGERGFHYGGGGGGSGGGGGIVEQCCTSTCSLDQLENYC

SEQ ID NO: 8 - protein, 58 aa, Artificial Sequence
  Insulin Polypeptide
FVNQHLCGSHLVEALELVCGERGFHYGGGGGGSGGGGGIVEQCCTSTCSLDQLENYCN

SEQ ID NO: 9 - protein, 57 aa, Artificial Sequence
  Insulin Polypeptide
  Xaa (10)..(10): Xaa is not D
  Xaa (45)..(45): Xaa is not H
FVNQHLCGSXLVEALALVCGERGFHYGGGGGGSGGGGGIVEQCCXSTCSLDQLENYC

SEQ ID NO: 10 - protein, 57 aa, Artificial Sequence
  Insulin Polypeptide
FVNQHLCGSHLVEALALVCGERGFHYGGGGGGSGGGGGIVEQCCTSTCSLDQLENYC

SEQ ID NO: 11 - protein, 9 aa, Artificial Sequence
  Linker
GGGGAGGGG

SEQ ID NO: 12 - protein, 9 aa, Artificial Sequence
  Linker
GGGGSGGGG

SEQ ID NO: 13 - protein, 21 aa, Artificial Sequence
  Linker
GGGGGQGGGGQGGGGQGGGGG

SEQ ID NO: 14 - protein, 228 aa, Artificial Sequence
  Fc Fragment dIgGA
RCTDTPPCPVPEPLGGPSVLIFPPKPKDILRITRTPEVTCVVLDLGREDPEVQISWFVDGKEVHTAKTQSREQQFNGTYRVVSVLPIEHQDWLTGKEFKCRVNHIDLPSPIERTISKARGRAHKPSVYVLPPSPKELSSSDTVSITCLIKDFYPPDIDVEWQSNGQQEPERKHRMTPPQLDEDGSYFLYSKLSVDKSRWQQGDPFTCAVMHETLQNHYTDLSLSHSPG

SEQ ID NO: 15 - protein, 224 aa, Artificial Sequence
  Fc Fragment dIgGB
DCPKCPAPEMLGGPSVFIFPPKPKDTLLIARTPEVTCVVVDLDPEDPEVQISWFVDGKQMQTAKTQPREEQFNGTYRVVSVLPIGHQDWLKGKQFTCKVNNKALPSPIERTISKARGQAHQPSVYVLPPSREELSKNTVSLTCLIKDFFPPDIDVEWQSNGQQEPESKYRTTPPQLDEDGSYFLYSKLSVDKSRWQRGDTFICAVMHEALHNHYTQESLSHSPG

SEQ ID NO: 16 - protein, 225 aa, Artificial Sequence
  Fc Fragment dIgGC
CNNCPCPGCGLLGGPSVFIFPPKPKDILVTARTPTVTCVVVDLDPENPEVQISWFVDSKQVQTANTQPREEQSNGTYRVVSVLPIGHQDWLSGKQFKCKVNNKALPSPIEEIISKTPGQAHQPNVYVLPPSRDEMSKNTVTLTCLVKDFFPPEIDVEWQSNGQQEPESKYRMTPPQLDEDGSYFLYSKLSVDKSRWQRGDTFICAVMHEALHNHYTQISLSHSPG

SEQ ID NO: 17 - protein, 225 aa, Artificial Sequence
  Fc Fragment dIgGD
CISPCPVPESLGGPSVFIFPPKPKDILRITRTPEITCVVLDLGREDPEVQISWFVDGKEVHTAKTQPREQQFNSTYRVVSVLPIEHQDWLTGKEFKCRVNHIGLPSPIERTISKARGQAHQPSVYVLPPSPKELSSSDTVTLTCLIKDFFPPEIDVEWQSNGQPEPESKYHTTAPQLDEDGSYFLYSKLSVDKSRWQQGDTFTCAVMHEALQNHYTDLSLSHSPG

SEQ ID NO: 18 - protein, 224 aa, Artificial Sequence
  Fc Fragment dIgGB-cNg-S
DCPKCPAPEMLGGPSVFIFPPKPKDTLLIARTPEVTCVVVDLDPEDPEVQISWFVDGKQMQTAKTQPREEQFSGTYRVVSVLPIGHQDWLKGKQFTCKVNNKALPSPIERTISKARGQAHQPSVYVLPPSREELSKNTVSLTCLIKDFFPPDIDVEWQSNGQQEPESKYRTTPPQLDEDGSYFLYSKLSVDKSRWQRGDTFICAVMHEALHNHYTQESLSHSPG

SEQ ID NO: 19 - protein, 9 aa, Artificial Sequence
  Linker
GGGGQGGGG

SEQ ID NO: 20 - protein, 303 aa, Artificial Sequence
  Insulin-Fc Fusion Protein
  Xaa (10)..(10): Xaa is not D
  Xaa (45)..(45): Xaa is not H
  Xaa (58)..(58): Xaa is absent or N
FVNQHLCGSXLVEALELVCGERGFHYGGGGGGSGGGGGIVEQCCXSTCSLDQLENYCXGGGGGQGGGGQGGGGQGGGGGDCPKCPAPEMLGGPSVFIFPPKPKDTLLIARTPEVTCVVVDLDPEDPEVQISWFVDGKQMQTAKTQPREEQFNGTYRVVSVLPIGHQDWLKGKQFTCKVNNKALPSPIERTISKARGQAHQPSVYVLPPSREELSKNTVSLTCLIKDFFPPDIDVEWQSNGQQEPESKYRTTPPQLDEDGSYFLYSKLSVDKSRWQRGDTFICAVMHEALHNHYTQESLSHSPG

SEQ ID NO: 21 - protein, 303 aa, Artificial Sequence
  Insulin-Fc Fusion Protein
  Xaa (58)..(58): Xaa is absent or N
FVNQHLCGSHLVEALELVCGERGFHYGGGGGGSGGGGGIVEQCCTSTCSLDQLENYCXGGGGGQGGGGQGGGGQGGGGGDCPKCPAPEMLGGPSVFIFPPKPKDTLLIARTPEVTCVVVDLDPEDPEVQISWFVDGKQMQTAKTQPREEQFNGTYRVVSVLPIGHQDWLKGKQFTCKVNNKALPSPIERTISKARGQAHQPSVYVLPPSREELSKNTVSLTCLIKDFFPPDIDVEWQSNGQQEPESKYRTTPPQLDEDGSYFLYSKLSVDKSRWQRGDTFICAVMHEALHNHYTQESLSHSPG

SEQ ID NO: 22 - protein, 302 aa, Artificial Sequence
  Insulin-Fc Fusion Protein
  Xaa (10)..(10): Xaa is not D
  Xaa (45)..(45): Xaa is not H
FVNQHLCGSXLVEALALVCGERGFHYGGGGGGSGGGGGIVEQCCXSTCSLDQLENYCGGGGGQGGGGQGGGGQGGGGGDCPKCPAPEMLGGPSVFIFPPKPKDTLLIARTPEVTCVVVDLDPEDPEVQISWFVDGKQMQTAKTQPREEQFSGTYRVVSVLPIGHQDWLKGKQFTCKVNNKALPSPIERTISKARGQAHQPSVYVLPPSREELSKNTVSLTCLIKDFFPPDIDVEWQSNGQQEPESKYRTTPPQLDEDGSYFLYSKLSVDKSRWQRGDTFICAVMHEALHNHYTQESLSHSPG

SEQ ID NO: 23 - DNA, 57 bp, Artificial Sequence
  Leader sequence cDNA
atggaatggagctgggtctttctcttcttcctgtcagtaacgactggtgtccactcc

SEQ ID NO: 24 - protein, 19 aa, Artificial Sequence
  Leader sequence
MEWSWVFLFFLSVTTGVHS

SEQ ID NO: 25 - DNA, 966 bp, Artificial Sequence
  cDNA for Insulin-Fc Fusion Protein
atggaatggagctgggtctttctcttcttcctgtcagtaacgactggtgtccactccttcgtgaaccagcacctgtgcggctcccacctggtggaagctctggaactcgtgtgcggcgagcggggcttccactacgggggtggcggaggaggttctggtggcggcggaggcatcgtggaacagtgctgcacctccacctgctccctggaccagctggaaaactactgcggtggcggaggtggtcaaggaggcggtggacagggtggaggtgggcagggaggaggcgggggagactgccccaagtgccccgctcccgagatgctgggcggacccagcgtgttcatcttccctcccaagcccaaggacacactgctgatcgccaggaccccggaggtgacctgcgtggtggtggacctggatcccgaagaccccgaggtgcagatcagctggttcgtggatggaaagcagatgcagaccgccaagacccaaccccgggaagagcagttcaacggcacctacagggtggtgagtgtgttgcccatcggccaccaggactggctgaaggggaagcaattcacatgcaaggttaataacaaggccctgcccagccccatcgagaggaccatcagcaaggccaggggccaggcccaccagccatctgtgtacgtgctgcccccatctagggaggaactgagcaagaacacagtcagccttacttgcctgatcaaggacttcttcccaccggacatagacgtggagtggcagagtaacggccagcaggagcccgagagcaagtataggaccacaccgccccaactggacgaggacggaagctacttcctctacagcaaattgagcgttgacaaaagcaggtggcagcgaggcgacaccttcatctgcgccgtgatgcacgaggctttgcataaccactacacccaggagagcctgtcccacagccccggatag

SEQ ID NO: 26 - protein, 302 aa, Artificial Sequence
  Insulin-Fc Fusion Protein
FVNQHLCGSHLVEALELVCGERGFHYGGGGGGSGGGGGIVEQCCTSTCSLDQLENYCGGGGGQGGGGQGGGGQGGGGGDCPKCPAPEMLGGPSVFIFPPKPKDTLLIARTPEVTCVVVDLDPEDPEVQISWFVDGKQMQTAKTQPREEQFNGTYRVVSVLPIGHQDWLKGKQFTCKVNNKALPSPIERTISKARGQAHQPSVYVLPPSREELSKNTVSLTCLIKDFFPPDIDVEWQSNGQQEPESKYRTTPPQLDEDGSYFLYSKLSVDKSRWQRGDTFICAVMHEALHNHYTQESLSHSPG

SEQ ID NO: 27 - DNA, 969 bp, Artificial Sequence
  cDNA for Insulin-Fc Fusion Protein
atggaatggagctgggtctttctcttcttcctgtcagtaacgactggtgtccactccttcgtgaaccagcacctgtgcggctcccacctggtggaagctctggaactcgtgtgcggcgagcggggcttccactacgggggtggcggaggaggttctggtggcggcggaggcatcgtggaacagtgctgcacctccacctgctccctggaccagctggaaaactactgcaacggtggcggaggtggtcaaggaggcggtggacagggtggaggtgggcagggaggaggcgggggagactgccccaagtgccccgctcccgagatgctgggcggacccagcgtgttcatcttccctcccaagcccaaggacacactgctgatcgccaggaccccggaggtgacctgcgtggtggtggacctggatcccgaagaccccgaggtgcagatcagctggttcgtggatggaaagcagatgcagaccgccaagacccaaccccgggaagagcagttcaacggcacctacagggtggtgagtgtgttgcccatcggccaccaggactggctgaaggggaagcaattcacatgcaaggttaataacaaggccctgcccagccccatcgagaggaccatcagcaaggccaggggccaggcccaccagccatctgtgtacgtgctgcccccatctagggaggaactgagcaagaacacagtcagccttacttgcctgatcaaggacttcttcccaccggacatagacgtggagtggcagagtaacggccagcaggagcccgagagcaagtataggaccacaccgccccaactggacgaggacggaagctacttcctctacagcaaattgagcgttgacaaaagcaggtggcagcgaggcgacaccttcatctgcgccgtgatgcacgaggctttgcataaccactacacccaggagagcctgtcccacagccccggatag

SEQ ID NO: 28 - protein, 303 aa, Artificial Sequence
  Insulin-Fc Fusion Protein
FVNQHLCGSHLVEALELVCGERGFHYGGGGGGSGGGGGIVEQCCTSTCSLDQLENYCNGGGGGQGGGGQGGGGQGGGGGDCPKCPAPEMLGGPSVFIFPPKPKDTLLIARTPEVTCVVVDLDPEDPEVQISWFVDGKQMQTAKTQPREEQFNGTYRVVSVLPIGHQDWLKGKQFTCKVNNKALPSPIERTISKARGQAHQPSVYVLPPSREELSKNTVSLTCLIKDFFPPDIDVEWQSNGQQEPESKYRTTPPQLDEDGSYFLYSKLSVDKSRWQRGDTFICAVMHEALHNHYTQESLSHSPG

SEQ ID NO: 29 - DNA, 966 bp, Artificial Sequence
  cDNA for Insulin-Fc Fusion Protein
atggaatggagctgggtctttctcttcttcctgtcagtaacgactggtgtccactccttcgtgaaccagcacctgtgcggctcccacctggtggaagctctggcactcgtgtgcggcgagcggggcttccactacgggggtggcggaggaggttctggtggcggcggaggcatcgtggaacagtgctgcacctccacctgctccctggaccagctggaaaactactgcggtggcggaggtggtcaaggaggcggtggacagggtggaggtgggcagggaggaggcgggggagactgccccaagtgccccgctcccgagatgctgggcggacccagcgtgttcatcttccctcccaagcccaaggacacactgctgatcgccaggaccccggaggtgacctgcgtggtggtggacctggatcccgaagaccccgaggtgcagatcagctggttcgtggatggaaagcagatgcagaccgccaagacccaaccccgggaagagcagttctcaggcacctacagggtggtgagtgtgttgcccatcggccaccaggactggctgaaggggaagcaattcacatgcaaggttaataacaaggccctgcccagccccatcgagaggaccatcagcaaggccaggggccaggcccaccagccatctgtgtacgtgctgcccccatctagggaggaactgagcaagaacacagtcagccttacttgcctgatcaaggacttcttcccaccggacatagacgtggagtggcagagtaacggccagcaggagcccgagagcaagtataggaccacaccgccccaactggacgaggacggaagctacttcctctacagcaaattgagcgttgacaaaagcaggtggcagcgaggcgacaccttcatctgcgccgtgatgcacgaggctttgcataaccactacacccaggagagcctgtcccacagccccggatag

SEQ ID NO: 30 - protein, 302 aa, Artificial Sequence
  Insulin-Fc Fusion Protein
FVNQHLCGSHLVEALALVCGERGFHYGGGGGGSGGGGGIVEQCCTSTCSLDQLENYCGGGGGQGGGGQGGGGQGGGGGDCPKCPAPEMLGGPSVFIFPPKPKDTLLIARTPEVTCVVVDLDPEDPEVQISWFVDGKQMQTAKTQPREEQFSGTYRVVSVLPIGHQDWLKGKQFTCKVNNKALPSPIERTISKARGQAHQPSVYVLPPSREELSKNTVSLTCLIKDFFPPDIDVEWQSNGQQEPESKYRTTPPQLDEDGSYFLYSKLSVDKSRWQRGDTFICAVMHEALHNHYTQESLSHSPG

SEQ ID NO: 31 - protein, 294 aa, Artificial Sequence
  Insulin-Fc Fusion Protein
FVNQHLCGSDLVEALALVCGERGFFYTDPTGGGPRRGIVEQCCHSICSLYQLENYCNGGGGAGGGGRCTDTPPCPVPEPLGGPSVLIFPPKPKDILRITRTPEVTCVVLDLGREDPEVQISWFVDGKEVHTAKTQSREQQFNGTYRVVSVLPIEHQDWLTGKEFKCRVNHIDLPSPIERTISKARGRAHKPSVYVLPPSPKELSSSDTVSITCLIKDFYPPDIDVEWQSNGQQEPERKHRMTPPQLDEDGSYFLYSKLSVDKSRWQQGDPFTCAVMHETLQNHYTDLSLSHSPG

SEQ ID NO: 32 - protein, 294 aa, Artificial Sequence
  Insulin-Fc Fusion Protein
FVNQHLCGSDLVEALALVCGERGFFYTDPTGGGPRRGIVEQCCHSICSLYQLENYCNGGGGAGGGGRCTDTPPCPVPEPLGGPSVLIFPPKPKDILRITRTPEVTCVVLDLGREDPEVQISWFVDGKEVHTAKTQSREQQFNGTYRVVSVLPIEHQDWLTGKEFKCRVNHIDLPSPIERTISKARGRAHKPSVYVLPPSPKELSSSDTVSITCLIKDFYPPDIDVEWQSNGQQEPERKHRMTPPQLDEDGSYFLYSKLSVDKSRWQQGDPFTCAVLHEALHSHYTQKSLSLSPG

SEQ ID NO: 33 - protein, 294 aa, Artificial Sequence
  Insulin-Fc Fusion Protein
FVNQHLCGSDLVEALALVCGERGFFYTDPTGGGPRRGIVEQCCHSICSLYQLENYCNGGGGAGGGGRCTDTPPCPVPEPLGGPSVLIFPPKPKDILRITRTPEVTCVVLDLGREDPEVQISWFVDGKEVHTAKTQSREQQFNGTYRVVSVLPIEHQDWLTGKEFKCRVNHIDLPSPIERTISKARGRAHKPSVYVLPPSPKELSSSDTVSITCLIKDFYPPDIDVEWQSNGQQEPERKHRMTPPQLDEDGSYFLYSKLSVDKSRWQQGDPFTCAVLHETLQSHYTDLSLSHSPG

SEQ ID NO: 34 - protein, 294 aa, Artificial Sequence
  Insulin-Fc Fusion Protein
FVNQHLCGSDLVEALALVCGERGFFYTDPTGGGPRRGIVEQCCHSICSLYQLENYCNGGGGAGGGGRCTDTPPCPVPEPLGGPSVLIFPPKPKDILRITRTPEVTCVVLDLGREDPEVQISWFVDGKEVHTAKTQSREQQFNGTYRVVSVLPIEHQDWLTGKEFKCRVNHIDLPSPIERTISKARGRAHKPSVYVLPPSPKELSSSDTVSITCLIKDFYPPDIDVEWQSNGQQEPERKHRMTPPQLDEDGSYFLYSKLSVDKSRWQQGDPFTCAVMHETLQSHYTDLSLSHSPG

SEQ ID NO: 35 - protein, 294 aa, Artificial Sequence
  Insulin-Fc Fusion Protein
FVNQHLCGSDLVEALALVCGERGFFYTDPTGGGPRRGIVEQCCHSICSLYQLENYCNGGGGAGGGGRCTDTPPCPVPEPLGGPSVLIFPPKPKDILRITRTPEVTCVVLDLGREDPEVQISWFVDGKEVHTAKTQSREQQFNGTYRVVSVLPIEHQDWLTGKEFKCRVNHIDLPSPIERTISKARGRAHKPSVYVLPPSPKELSSSDTVSITCLIKDFYPPDIDVEWQSNGQQEPERKHRMTPPQLDEDGSYFLYSKLSVDKSRWQQGDPFTCAVLHETLQNHYTDLSLSHSPG

SEQ ID NO: 36 - protein, 290 aa, Artificial Sequence
  Insulin-Fc Fusion Protein
FVNQHLCGSDLVEALALVCGERGFFYTDPTGGGPRRGIVEQCCHSICSLYQLENYCNGGGGAGGGGDCPKCPAPEMLGGPSVFIFPPKPKDTLLIARTPEVTCVVVDLDPEDPEVQISWFVDGKQMQTAKTQPREEQFNGTYRVVSVLPIGHQDWLKGKQFTCKVNNKALPSPIERTISKARGQAHQPSVYVLPPSREELSKNTVSLTCLIKDFFPPDIDVEWQSNGQQEPESKYRTTPPQLDEDGSYFLYSKLSVDKSRWQRGDTFICAVMHEALHNHYTQESLSHSPG

SEQ ID NO: 37 - protein, 291 aa, Artificial Sequence
  Insulin-Fc Fusion Protein
FVNQHLCGSDLVEALALVCGERGFFYTDPTGGGPRRGIVEQCCHSICSLYQLENYCNGGGGAGGGGCNNCPCPGCGLLGGPSVFIFPPKPKDILVTARTPTVTCVVVDLDPENPEVQISWFVDSKQVQTANTQPREEQSNGTYRVVSVLPIGHQDWLSGKQFKCKVNNKALPSPIEEIISKTPGQAHQPNVYVLPPSRDEMSKNTVTLTCLVKDFFPPEIDVEWQSNGQQEPESKYRMTPPQLDEDGSYFLYSKLSVDKSRWQRGDTFICAVMHEALHNHYTQISLSHSPG

SEQ ID NO: 38 - protein, 291 aa, Artificial Sequence
  Insulin-Fc Fusion Protein
FVNQHLCGSDLVEALALVCGERGFFYTDPTGGGPRRGIVEQCCHSICSLYQLENYCNGGGGAGGGGCISPCPVPESLGGPSVFIFPPKPKDILRITRTPEITCVVLDLGREDPEVQISWFVDGKEVHTAKTQPREQQFNSTYRVVSVLPIEHQDWLTGKEFKCRVNHIGLPSPIERTISKARGQAHQPSVYVLPPSPKELSSSDTVTLTCLIKDFFPPEIDVEWQSNGQPEPESKYHTTAPQLDEDGSYFLYSKLSVDKSRWQQGDTFTCAVMHEALQNHYTDLSLSHSPG

SEQ ID NO: 39 - protein, 290 aa, Artificial Sequence
  Insulin-Fc Fusion Protein
FVNQHLCGSDLVEALALVCGERGFFYTDPTGGGPRRGIVEQCCHSICSLYQLENYCNGGGGAGGGGDCPKCPAPEMLGGPSVFIFPPKPKDTLLIARTPEVTCVVVDLDPEDPEVQISWFVDGKQMQTAKTQPREEQFQGTYRVVSVLPIGHQDWLKGKQFTCKVNNKALPSPIERTISKARGQAHQPSVYVLPPSREELSKNTVSLTCLIKDFFPPDIDVEWQSNGQQEPESKYRTTPPQLDEDGSYFLYSKLSVDKSRWQRGDTFICAVMHEALHNHYTQESLSHSPG

SEQ ID NO: 40 - protein, 290 aa, Artificial Sequence
  Insulin-Fc Fusion Protein
FVNQHLCGSDLVEALALVCGERGFFYTDPTGGGPRRGIVEQCCHSICSLYQLENYCNGGGGAGGGGDCPKCPAPEMLGGPSVFIFPPKPKDTLLIARTPEVTCVVVDLDPEDPEVQISWFVDGKQMQTAKTQPREEQFSGTYRVVSVLPIGHQDWLKGKQFTCKVNNKALPSPIERTISKARGQAHQPSVYVLPPSREELSKNTVSLTCLIKDFFPPDIDVEWQSNGQQEPESKYRTTPPQLDEDGSYFLYSKLSVDKSRWQRGDTFICAVMHEALHNHYTQESLSHSPG

SEQ ID NO: 41 - protein, 290 aa, Artificial Sequence
  Insulin-Fc Fusion Protein
FVNQHLCGSDLVEALALVCGERGFFYTDPTGGGPRRGIVEQCCHSICSLYQLENYCNGGGGAGGGGDCPKCPAPEMLGGPSVFIFPPKPKDTLLIARTPEVTCVVVDLDPEDPEVQISWFVDGKQMQTAKTQPREEQFDGTYRVVSVLPIGHQDWLKGKQFTCKVNNKALPSPIERTISKARGQAHQPSVYVLPPSREELSKNTVSLTCLIKDFFPPDIDVEWQSNGQQEPESKYRTTPPQLDEDGSYFLYSKLSVDKSRWQRGDTFICAVMHEALHNHYTQESLSHSPG

SEQ ID NO: 42 - protein, 290 aa, Artificial Sequence
  Insulin-Fc Fusion Protein
FVNQHLCGSDLVEALALVCGERGFFYTDPTGGGPRRGIVEQCCHSICSLYQLENYCNGGGGAGGGGDCPKCPAPEMLGGPSVFIFPPKPKDTLLIARTPEVTCVVVDLDPEDPEVQISWFVDGKQMQTAKTQPREEQFKGTYRVVSVLPIGHQDWLKGKQFTCKVNNKALPSPIERTISKARGQAHQPSVYVLPPSREELSKNTVSLTCLIKDFFPPDIDVEWQSNGQQEPESKYRTTPPQLDEDGSYFLYSKLSVDKSRWQRGDTFICAVMHEALHNHYTQESLSHSPG

SEQ ID NO: 43 - protein, 290 aa, Artificial Sequence
  Insulin-Fc Fusion Protein
FVNQHLCGSHLVEALALVCGERGFFYTDPTGGGPRRGIVEQCCTSICSLYQLENYCNGGGGAGGGGDCPKCPAPEMLGGPSVFIFPPKPKDTLLIARTPEVTCVVVDLDPEDPEVQISWFVDGKQMQTAKTQPREEQFQGTYRVVSVLPIGHQDWLKGKQFTCKVNNKALPSPIERTISKARGQAHQPSVYVLPPSREELSKNTVSLTCLIKDFFPPDIDVEWQSNGQQEPESKYRTTPPQLDEDGSYFLYSKLSVDKSRWQRGDTFICAVMHEALHNHYTQESLSHSPG

SEQ ID NO: 44 - protein, 289 aa, Artificial Sequence
  Insulin-Fc Fusion Protein
FVNQHLCGSHLVQALYLVCGERGFFYTDPTGGGPRRGIVEQCCTSICSLYQLENYCGGGGAGGGGDCPKCPAPEMLGGPSVFIFPPKPKDTLLIARTPEVTCVVVDLDPEDPEVQISWFVDGKQMQTAKTQPREEQFSGTYRVVSVLPIGHQDWLKGKQFTCKVNNKALPSPIERTISKARGQAHQPSVYVLPPSREELSKNTVSLTCLIKDFFPPDIDVEWQSNGQQEPESKYRTTPPQLDEDGSYFLYSKLSVDKSRWQRGDTFICAVMHEALHNHYTQESLSHSPG

SEQ ID NO: 45 - protein, 289 aa, Artificial Sequence
  Insulin-Fc Fusion Protein
FVNQHLCGSELVEALALVCGERGFFYTDPTGGGPRRGIVEQCCTSICSLYQLENYCGGGGAGGGGDCPKCPAPEMLGGPSVFIFPPKPKDTLLIARTPEVTCVVVDLDPEDPEVQISWFVDGKQMQTAKTQPREEQFSGTYRVVSVLPIGHQDWLKGKQFTCKVNNKALPSPIERTISKARGQAHQPSVYVLPPSREELSKNTVSLTCLIKDFFPPDIDVEWQSNGQQEPESKYRTTPPQLDEDGSYFLYSKLSVDKSRWQRGDTFICAVMHEALHNHYTQESLSHSPG

SEQ ID NO: 46 - protein, 289 aa, Artificial Sequence
  Insulin-Fc Fusion Protein
FVNQHLCGSHLVEALALVCGEAGFFYTDPTGGGPRRGIVEQCCTSICSLYQLENYCGGGGAGGGGDCPKCPAPEMLGGPSVFIFPPKPKDTLLIARTPEVTCVVVDLDPEDPEVQISWFVDGKQMQTAKTQPREEQFSGTYRVVSVLPIGHQDWLKGKQFTCKVNNKALPSPIERTISKARGQAHQPSVYVLPPSREELSKNTVSLTCLIKDFFPPDIDVEWQSNGQQEPESKYRTTPPQLDEDGSYFLYSKLSVDKSRWQRGDTFICAVMHEALHNHYTQESLSHSPG

SEQ ID NO: 47 - protein, 289 aa, Artificial Sequence
  Insulin-Fc Fusion Protein
FVNQHLCGSHLVEALALVCGERGFYYTDPTGGGPRRGIVEQCCTSICSLYQLENYCGGGGAGGGGDCPKCPAPEMLGGPSVFIFPPKPKDTLLIARTPEVTCVVVDLDPEDPEVQISWFVDGKQMQTAKTQPREEQFSGTYRVVSVLPIGHQDWLKGKQFTCKVNNKALPSPIERTISKARGQAHQPSVYVLPPSREELSKNTVSLTCLIKDFFPPDIDVEWQSNGQQEPESKYRTTPPQLDEDGSYFLYSKLSVDKSRWQRGDTFICAVMHEALHNHYTQESLSHSPG

SEQ ID NO: 48 - protein, 289 aa, Artificial Sequence
  Insulin-Fc Fusion Protein
FVNQHLCGSHLVEALALVCGERGFFYTDPTGGGPRRGIVEQCCTSICSLYQLENYCGGGGAGGGGDCPKCPAPEMLGGPSVFIFPPKPKDTLLIARTPEVTCVVVDLDPEDPEVQISWFVDGKQMQTAKTQPREEQFSGTYRVVSVLPIGHQDWLKGKQFTCKVNNKALPSPIERTISKARGQAHQPSVYVLPPSREELSKNTVSLTCLIKDFFPPDIDVEWQSNGQQEPESKYRTTPPQLDEDGSYFLYSKLSVDKSRWQRGDTFICAVMHEALHNHYTQESLSHSPG

SEQ ID NO: 49 - protein, 292 aa, Artificial Sequence
  Insulin-Fc Fusion Protein
FVNQHLCGSHLVQALYLVCGERGFFYTDPTQRGGGGGQRGIVEQCCTSICSLYQLENYCGGGGAGGGGDCPKCPAPEMLGGPSVFIFPPKPKDTLLIARTPEVTCVVVDLDPEDPEVQISWFVDGKQMQTAKTQPREEQFSGTYRVVSVLPIGHQDWLKGKQFTCKVNNKALPSPIERTISKARGQAHQPSVYVLPPSREELSKNTVSLTCLIKDFFPPDIDVEWQSNGQQEPESKYRTTPPQLDEDGSYFLYSKLSVDKSRWQRGDTFICAVMHEALHNHYTQESLSHSPG

SEQ ID NO: 50 - protein, 294 aa, Artificial Sequence
  Insulin-Fc Fusion Protein
FVNQHLCGSHLVEALALVCGERGFFYTDPTGGGGGGSGGGGGIVEQCCTSICSLYQLENYCGGGGAGGGGDCPKCPAPEMLGGPSVFIFPPKPKDTLLIARTPEVTCVVVDLDPEDPEVQISWFVDGKQMQTAKTQPREEQFSGTYRVVSVLPIGHQDWLKGKQFTCKVNNKALPSPIERTISKARGQAHQPSVYVLPPSREELSKNTVSLTCLIKDFFPPDIDVEWQSNGQQEPESKYRTTPPQLDEDGSYFLYSKLSVDKSRWQRGDTFICAVMHEALHNHYTQESLSHSPG

SEQ ID NO: 51 - protein, 290 aa, Artificial Sequence
  Insulin-Fc Fusion Protein
FVNQHLCGSHLVEALALVCGERGFFYTDPGGGGGGGGGIVEQCCTSICSLYQLENYCGGGGAGGGGDCPKCPAPEMLGGPSVFIFPPKPKDTLLIARTPEVTCVVVDLDPEDPEVQISWFVDGKQMQTAKTQPREEQFSGTYRVVSVLPIGHQDWLKGKQFTCKVNNKALPSPIERTISKARGQAHQPSVYVLPPSREELSKNTVSLTCLIKDFFPPDIDVEWQSNGQQEPESKYRTTPPQLDEDGSYFLYSKLSVDKSRWQRGDTFICAVMHEALHNHYTQESLSHSPG

SEQ ID NO: 52 - protein, 289 aa, Artificial Sequence
  Insulin-Fc Fusion Protein
FVNQHLCGSHLVEALALVCGERGFFYTPGGGGGGGGGIVEQCCTSICSLYQLENYCGGGGAGGGGDCPKCPAPEMLGGPSVFIFPPKPKDTLLIARTPEVTCVVVDLDPEDPEVQISWFVDGKQMQTAKTQPREEQFSGTYRVVSVLPIGHQDWLKGKQFTCKVNNKALPSPIERTISKARGQAHQPSVYVLPPSREELSKNTVSLTCLIKDFFPPDIDVEWQSNGQQEPESKYRTTPPQLDEDGSYFLYSKLSVDKSRWQRGDTFICAVMHEALHNHYTQESLSHSPG

SEQ ID NO: 53 - protein, 301 aa, Artificial Sequence
  Insulin-Fc Fusion Protein
FVNQHLCGSHLVEALALVCGERGFFYTDPTGGGPRRGIVEQCCTSICSLYQLENYCGGGGGQGGGGQGGGGQGGGGGDCPKCPAPEMLGGPSVFIFPPKPKDTLLIARTPEVTCVVVDLDPEDPEVQISWFVDGKQMQTAKTQPREEQFSGTYRVVSVLPIGHQDWLKGKQFTCKVNNKALPSPIERTISKARGQAHQPSVYVLPPSREELSKNTVSLTCLIKDFFPPDIDVEWQSNGQQEPESKYRTTPPQLDEDGSYFLYSKLSVDKSRWQRGDTFICAVMHEALHNHYTQESLSHSPG

SEQ ID NO: 54 - protein, 289 aa, Artificial Sequence
  Insulin-Fc Fusion Protein
FVNQHLCGSHLVEALALVCGERGFFYTQGGGGGGGGGIVEQCCTSICSLYQLENYCGGGGAGGGGDCPKCPAPEMLGGPSVFIFPPKPKDTLLIARTPEVTCVVVDLDPEDPEVQISWFVDGKQMQTAKTQPREEQFSGTYRVVSVLPIGHQDWLKGKQFTCKVNNKALPSPIERTISKARGQAHQPSVYVLPPSREELSKNTVSLTCLIKDFFPPDIDVEWQSNGQQEPESKYRTTPPQLDEDGSYFLYSKLSVDKSRWQRGDTFICAVMHEALHNHYTQESLSHSPG

SEQ ID NO: 55 - protein, 302 aa, Artificial Sequence
  Insulin-Fc Fusion Protein
FVNQHLCGSHLVEALELVCGERGFFYTPKTGGSGGGGGIVEQCCTSTCSLDQLENYCGGGGGQGGGGQGGGGQGGGGGDCPKCPAPEMLGGPSVFIFPPKPKDTLLIARTPEVTCVVVDLDPEDPEVQISWFVDGKQMQTAKTQPREEQFNGTYRVVSVLPIGHQDWLKGKQFTCKVNNKALPSPIERTISKARGQAHQPSVYVLPPSREELSKNTVSLTCLIKDFFPPDIDVEWQSNGQQEPESKYRTTPPQLDEDGSYFLYSKLSVDKSRWQRGDTFICAVMHEALHNHYTQESLSHSPG

SEQ ID NO: 56 - protein, 303 aa, Artificial Sequence
  Insulin-Fc Fusion Protein
FVNQHLCGSHLVEALELVCGERGFHYGGGGGGSGGGGGIVEQCCTSTCSLDQLENYCNHGGGGQGGGGQGGGGQGGGGGDCPKCPAPEMLGGPSVFIFPPKPKDTLLIARTPEVTCVVVDLDPEDPEVQISWFVDGKQMQTAKTQPREEQFNGTYRVVSVLPIGHQDWLKGKQFTCKVNNKALPSPIERTISKARGQAHQPSVYVLPPSREELSKNTVSLTCLIKDFFPPDIDVEWQSNGQQEPESKYRTTPPQLDEDGSYFLYSKLSVDKSRWQRGDTFICAVMHEALHNHYTQESLSHSPG

SEQ ID NO: 57 - protein, 302 aa, Artificial Sequence
  Insulin-Fc Fusion Protein
FVNQHLCGSHLVEALELVCGERGFFYGGGGGGSGGGGGIVEQCCTSTCSLDQLENYCGGGGGQGGGGQGGGGQGGGGGDCPKCPAPEMLGGPSVFIFPPKPKDTLLIARTPEVTCVVVDLDPEDPEVQISWFVDGKQMQTAKTQPREEQFNGTYRVVSVLPIGHQDWLKGKQFTCKVNNKALPSPIERTISKARGQAHQPSVYVLPPSREELSKNTVSLTCLIKDFFPPDIDVEWQSNGQQEPESKYRTTPPQLDEDGSYFLYSKLSVDKSRWQRGDTFICAVMHEALHNHYTQESLSHSPG

SEQ ID NO: 58 - protein, 306 aa, Artificial Sequence
  Insulin-Fc Fusion Protein
FVNQHLCGSHLVEALELVCGERGFHYGGGGGGSGGGGGIVEQCCTSTCSLDQLENYCGGGGGQGGGGQGGGGQGGGGGRCTDTPPCPVPEPLGGPSVLIFPPKPKDILRITRTPEVTCVVLDLGREDPEVQISWFVDGKEVHTAKTQSREQQFNGTYRVVSVLPIEHQDWLTGKEFKCRVNHIDLPSPIERTISKARGRAHKPSVYVLPPSPKELSSSDTVSITCLIKDFYPPDIDVEWQSNGQQEPERKHRMTPPQLDEDGSYFLYSKLSVDKSRWQQGDPFTCAVMHETLQNHYTDLSLSHSPG

SEQ ID NO: 59 - protein, 303 aa, Artificial Sequence
  Insulin-Fc Fusion Protein
FVNQHLCGSHLVEALELVCGERGFHYGGGGGGSGGGGGIVEQCCTSTCSLDQLENYCGGGGGQGGGGQGGGGQGGGGGCNNCPCPGCGLLGGPSVFIFPPKPKDILVTARTPTVTCVVVDLDPENPEVQISWFVDSKQVQTANTQPREEQSNGTYRVVSVLPIGHQDWLSGKQFKCKVNNKALPSPIEEIISKTPGQAHQPNVYVLPPSRDEMSKNTVTLTCLVKDFFPPEIDVEWQSNGQQEPESKYRMTPPQLDEDGSYFLYSKLSVDKSRWQRGDTFICAVMHEALHNHYTQISLSHSPG

SEQ ID NO: 60 - protein, 303 aa, Artificial Sequence
  Insulin-Fc Fusion Protein
FVNQHLCGSHLVEALELVCGERGFHYGGGGGGSGGGGGIVEQCCTSTCSLDQLENYCGGGGGQGGGGQGGGGQGGGGGCISPCPVPESLGGPSVFIFPPKPKDILRITRTPEITCVVLDLGREDPEVQISWFVDGKEVHTAKTQPREQQFNSTYRVVSVLPIEHQDWLTGKEFKCRVNHIGLPSPIERTISKARGQAHQPSVYVLPPSPKELSSSDTVTLTCLIKDFFPPEIDVEWQSNGQPEPESKYHTTAPQLDEDGSYFLYSKLSVDKSRWQQGDTFTCAVMHEALQNHYTDLSLSHSPG

SEQ ID NO: 61 - protein, 302 aa, Artificial Sequence
  Insulin-Fc Fusion Protein
FVNQHLCGSHLVEALELVCGERGFHYGGGGGGSGGGGGIVEQCCTSTCSLDQLENYCGGGGGQGGGGQGGGGQGGGGGDCPKCPAPEMLGGPSVFIFPPKPKDTLLIARTPEVTCVVVALDPEDPEVQISWFVDGKQMQTAKTQPREEQFSGTYRVVSVLPIGHQDWLKGKQFTCKVNNKALPSPIERTISKARGQAHQPSVYVLPPSREELSKNTVSLTCLIKDFFPPDIDVEWQSNGQQEPESKYRTTPPQLDEDGSYFLYSKLSVDKSRWQRGDTFICAVMHEALHNHYTQESLSHSPG

SEQ ID NO: 62 - protein, 302 aa, Artificial Sequence
  Insulin-Fc Fusion Protein
FVNQHLCGSHLVEALELVCGERGFHYGGGGGGSGGGGGIVEQCCTSTCSLDQLENYCGGGGGQGGGGQGGGGQGGGGGDCPKCPAPEMLGGPSVFIFPPKPKDTLLIARTPEVTCVVVDLDPEDPEVQISWFVDGKQMQTAKTQPREEQFSGTYRVVSVLPIGHQDWLKGKQFTCKVNNKALPSPIERTISKARGQAHQPSVYVLPPSREELSKNTVSLTCLIKDFFPPDIDVEWQSNGQQEPESKYRTTPPQLDEDGSYFLYSKLSVDKSRWQRGDTFICAVMHEALHNHYTQESLSHSPG

SEQ ID NO: 63 - protein, 57 aa, Artificial Sequence
  Insulin Polypeptide
FVNQHLCGSHLVEALALVCGERGFFYTDPTGGGPRRGIVEQCCTSICSLYQLENYCN

SEQ ID NO: 64 - protein, 10 aa, Artificial Sequence
  Linker
GGGGGAGGGG

SEQ ID NO: 65 - protein, 19 aa, Artificial Sequence
  Linker
GGGGSGGGGSGGGGSGGGG

SEQ ID NO: 66 - protein, 19 aa, Artificial Sequence
  Linker
GGGGKGGGGKGGGGKGGGG

SEQ ID NO: 67 - protein, 21 aa, Artificial Sequence
  Linker
GGGGGAGGGGAGGGGAGGGGG

SEQ ID NO: 68 - protein, 21 aa, Artificial Sequence
  Linker
SGGGGQGGGGQGGGGQGGGGG

SEQ ID NO: 69 - protein, 21 aa, Artificial Sequence
  Linker
HGGGGQGGGGQGGGGQGGGGG

SEQ ID NO: 70 - protein, 22 aa, Artificial Sequence
  Linker
PGGGGGQGGGGQGGGGQGGGGG

SEQ ID NO: 71 - protein, 11 aa, Artificial Sequence
  C-Chain
GGGGGGSGGGG

SEQ ID NO: 72 - protein, 7 aa, Artificial Sequence
  C-Chain
GGSGGGG

SEQ ID NO: 73 - protein, 226 aa, Artificial Sequence
  Fc Fragment hIgG1
DKTHTCPPCPAPELLGGPSVFLFPPKPKDTLMISRTPEVTCVVVDVSHEDPEVKFNWYVDGVEVHNAKTKPREEQYNSTYRVVSVLTVLHQDWLNGKEYKCKVSNKALPAPIEKTISKAKGQPREPQVYTLPPSRDELTKNQVSLTCLVKGFYPSDIAVEWESNGQPENNYKTTPPVLDSDGSFFLYSKLTVDKSRWQQGNVFSCSVMHEALHNHYTQKSLSLSPG

SEQ ID NO: 74 - protein, 221 aa, Artificial Sequence
  Fc Fragment hIgG2
ECPPCPAPPVAGPSVFLFPPKPKDTLMISRTPEVTCVVVDVSHEDPEVQFNWYVDGVEVHNAKTKPREEQFNSTFRVVSVLTVVHQDWLNGKEYKCKVSNKGLPAPIEKTISKTKGQPREPQVYTLPPSREEMTKNQVSLTCLVKGFYPSDIAVEWESNGQPENNYKTTPPMLDSDGSFFLYSKLTVDKSRWQQGNVFSCSVMHEALHNHYTQKSLSLSPG

SEQ ID NO: 75 - protein, 299 aa, Artificial Sequence
  Insulin-Fc Fusion Protein
FVNQHLCGSHLVEALELVCGERGFHYGGGGGGSGGGGGIVEQCCTSTCSLDQLENYCGGGGGQGGGGQGGGGQGGGGGECPPCPAPPVAGPSVFLFPPKPKDTLMISRTPEVTCVVVDVSHEDPEVQFNWYVDGVEVHNAKTKPREEQFNSTFRVVSVLTVVHQDWLNGKEYKCKVSNKGLPAPIEKTISKTKGQPREPQVYTLPPSREEMTKNQVSLTCLVKGFYPSDIAVEWESNGQPENNYKTTPPMLDSDGSFFLYSKLTVDKSRWQQGNVFSCSVMHEALHNHYTQKSLSLSPG

SEQ ID NO: 76 - protein, 304 aa, Artificial Sequence
  Insulin-Fc Fusion Protein
FVNQHLCGSHLVEALELVCGERGFHYGGGGGGSGGGGGIVEQCCTSTCSLDQLENYCGGGGGQGGGGQGGGGQGGGGGDKTHTCPPCPAPELLGGPSVFLFPPKPKDTLMISRTPEVTCVVVDVSHEDPEVKFNWYVDGVEVHNAKTKPREEQYNSTYRVVSVLTVLHQDWLNGKEYKCKVSNKALPAPIEKTISKAKGQPREPQVYTLPPSRDELTKNQVSLTCLVKGFYPSDIAVEWESNGQPENNYKTTPPVLDSDGSFFLYSKLTVDKSRWQQGNVFSCSVMHEALHNHYTQKSLSLSPG

SEQ ID NO: 77 - protein, 226 aa, Artificial Sequence
  Fc Fragment hIgG1 Consensus
  Xaa (77)..(77): Xaa is S,D,A,R or Q
DKTHTCPPCPAPELLGGPSVFLFPPKPKDTLMISRTPEVTCVVVDVSHEDPEVKFNWYVDGVEVHNAKTKPREEQYXSTYRVVSVLTVLHQDWLNGKEYKCKVSNKALPAPIEKTISKAKGQPREPQVYTLPPSRDELTKNQVSLTCLVKGFYPSDIAVEWESNGQPENNYKTTPPVLDSDGSFFLYSKLTVDKSRWQQGNVFSCSVMHEALHNHYTQKSLSLSPG

SEQ ID NO: 78 - protein, 304 aa, Artificial Sequence
  Insulin-Fc Fusion Protein
FVNQHLCGSHLVEALALVCGERGFHYGGGGGGSGGGGGIVEQCCTSTCSLDQLENYCGGGGGQGGGGQGGGGQGGGGGDKTHTCPPCPAPELLGGPSVFLFPPKPKDTLMISRTPEVTCVVVDVSHEDPEVKFNWYVDGVEVHNAKTKPREEQYSSTYRVVSVLTVLHQDWLNGKEYKCKVSNKALPAPIEKTISKAKGQPREPQVYTLPPSRDELTKNQVSLTCLVKGFYPSDIAVEWESNGQPENNYKTTPPVLDSDGSFFLYSKLTVDKSRWQQGNVFSCSVMHEALHNHYTQKSLSLSPG

SEQ ID NO: 79 - DNA, 972 bp, Artificial Sequence
  cDNA for Insulin-Fc Fusion Protein
atggaatggagctgggtctttctcttcttcctgtcagtaacgactggtgtccactccttcgtgaaccagcacctgtgcggctcccacctggtggaagctctggcactcgtgtgcggcgagcggggcttccactacgggggtggcggaggaggttctggtggcggcggaggcatcgtggaacagtgctgcacctccacctgctccctggaccagctggaaaactactgcggtggcggaggtggtcaaggaggcggtggacagggtggaggtgggcagggaggaggcgggggagacaaaactcacacatgcccaccgtgcccagcacctgaactcctggggggaccgtcagtcttcctcttccccccaaaacccaaggacaccctcatgatctcccggacccctgaggtcacatgcgtggtggtggacgtgagccacgaagaccctgaggtcaagttcaactggtacgtggacggcgtggaggtgcataatgccaagacaaagccgcgggaggagcagtacagcagcacgtaccgtgtggtcagcgtcctcaccgtcctgcaccaggactggctgaatggcaaggagtacaagtgcaaggtctccaacaaagccctcccagcccccatcgagaaaaccatctccaaagccaaagggcagccccgagaaccacaggtgtacaccctgcccccatcccgggatgagctgaccaagaaccaggtcagcctgacctgcctggtcaaaggcttctatcccagcgacatcgccgtggagtgggagagcaatgggcagccggagaacaactacaagaccacgcctcccgtgctggactccgacggctccttcttcctctacagcaagctcaccgtggacaagagcaggtggcagcaggggaacgtcttctcatgctccgtgatgcatgaggctctgcacaaccactacacgcagaagagcctctccctgtctccgggttag

SEQ ID NO: 80 - protein, 304 aa, Artificial Sequence
  Insulin-Fc Fusion Protein
FVNQHLCGSHLVEALALVCGERGFHYGGGGGGSGGGGGIVEQCCTSTCSLDQLENYCGGGGGQGGGGQGGGGQGGGGGDKTHTCPPCPAPELLGGPSVFLFPPKPKDTLMISRTPEVTCVVVDVSHEDPEVKFNWYVDGVEVHNAKTKPREEQYDSTYRVVSVLTVLHQDWLNGKEYKCKVSNKALPAPIEKTISKAKGQPREPQVYTLPPSRDELTKNQVSLTCLVKGFYPSDIAVEWESNGQPENNYKTTPPVLDSDGSFFLYSKLTVDKSRWQQGNVFSCSVMHEALHNHYTQKSLSLSPG

SEQ ID NO: 81 - DNA, 972 bp, Artificial Sequence
  cDNA for Insulin-Fc Fusion Protein
atggaatggagctgggtctttctcttcttcctgtcagtaacgactggtgtccactccttcgtgaaccagcacctgtgcggctcccacctggtggaagctctggcactcgtgtgcggcgagcggggcttccactacgggggtggcggaggaggttctggtggcggcggaggcatcgtggaacagtgctgcacctccacctgctccctggaccagctggaaaactactgcggtggcggaggtggtcaaggaggcggtggacagggtggaggtgggcagggaggaggcgggggagacaaaactcacacatgcccaccgtgcccagcacctgaactcctggggggaccgtcagtcttcctcttccccccaaaacccaaggacaccctcatgatctcccggacccctgaggtcacatgcgtggtggtggacgtgagccacgaagaccctgaggtcaagttcaactggtacgtggacggcgtggaggtgcataatgccaagacaaagccgcgggaggagcagtacgacagcacgtaccgtgtggtcagcgtcctcaccgtcctgcaccaggactggctgaatggcaaggagtacaagtgcaaggtctccaacaaagccctcccagcccccatcgagaaaaccatctccaaagccaaagggcagccccgagaaccacaggtgtacaccctgcccccatcccgggatgagctgaccaagaaccaggtcagcctgacctgcctggtcaaaggcttctatcccagcgacatcgccgtggagtgggagagcaatgggcagccggagaacaactacaagaccacgcctcccgtgctggactccgacggctccttcttcctctacagcaagctcaccgtggacaagagcaggtggcagcaggggaacgtcttctcatgctccgtgatgcatgaggctctgcacaaccactacacgcagaagagcctctccctgtctccgggttag

SEQ ID NO: 82 - protein, 304 aa, Artificial Sequence
  Insulin-Fc Fusion Protein
FVNQHLCGSHLVEALALVCGERGFHYGGGGGGSGGGGGIVEQCCTSTCSLDQLENYCGGGGGQGGGGQGGGGQGGGGGDKTHTCPPCPAPELLGGPSVFLFPPKPKDTLMISRTPEVTCVVVDVSHEDPEVKFNWYVDGVEVHNAKTKPREEQYASTYRVVSVLTVLHQDWLNGKEYKCKVSNKALPAPIEKTISKAKGQPREPQVYTLPPSRDELTKNQVSLTCLVKGFYPSDIAVEWESNGQPENNYKTTPPVLDSDGSFFLYSKLTVDKSRWQQGNVFSCSVMHEALHNHYTQKSLSLSPG

SEQ ID NO: 83 - DNA, 972 bp, Artificial Sequence
  cDNA for Insulin-Fc Fusion Protein
atggaatggagctgggtctttctcttcttcctgtcagtaacgactggtgtccactccttcgtgaaccagcacctgtgcggctcccacctggtggaagctctggcactcgtgtgcggcgagcggggcttccactacgggggtggcggaggaggttctggtggcggcggaggcatcgtggaacagtgctgcacctccacctgctccctggaccagctggaaaactactgcggtggcggaggtggtcaaggaggcggtggacagggtggaggtgggcagggaggaggcgggggagacaaaactcacacatgcccaccgtgcccagcacctgaactcctggggggaccgtcagtcttcctcttccccccaaaacccaaggacaccctcatgatctcccggacccctgaggtcacatgcgtggtggtggacgtgagccacgaagaccctgaggtcaagttcaactggtacgtggacggcgtggaggtgcataatgccaagacaaagccgcgggaggagcagtacgccagcacgtaccgtgtggtcagcgtcctcaccgtcctgcaccaggactggctgaatggcaaggagtacaagtgcaaggtctccaacaaagccctcccagcccccatcgagaaaaccatctccaaagccaaagggcagccccgagaaccacaggtgtacaccctgcccccatcccgggatgagctgaccaagaaccaggtcagcctgacctgcctggtcaaaggcttctatcccagcgacatcgccgtggagtgggagagcaatgggcagccggagaacaactacaagaccacgcctcccgtgctggactccgacggctccttcttcctctacagcaagctcaccgtggacaagagcaggtggcagcaggggaacgtcttctcatgctccgtgatgcatgaggctctgcacaaccactacacgcagaagagcctctccctgtctccgggttag

SEQ ID NO: 84 - protein, 304 aa, Artificial Sequence
  Insulin-Fc Fusion Protein
FVNQHLCGSHLVEALALVCGERGFHYGGGGGGSGGGGGIVEQCCTSTCSLDQLENYCGGGGGQGGGGQGGGGQGGGGGDKTHTCPPCPAPELLGGPSVFLFPPKPKDTLMISRTPEVTCVVVDVSHEDPEVKFNWYVDGVEVHNAKTKPREEQYRSTYRVVSVLTVLHQDWLNGKEYKCKVSNKALPAPIEKTISKAKGQPREPQVYTLPPSRDELTKNQVSLTCLVKGFYPSDIAVEWESNGQPENNYKTTPPVLDSDGSFFLYSKLTVDKSRWQQGNVFSCSVMHEALHNHYTQKSLSLSPG

SEQ ID NO: 85 - DNA, 972 bp, Artificial Sequence
  cDNA for Insulin-Fc Fusion Protein
atggaatggagctgggtctttctcttcttcctgtcagtaacgactggtgtccactccttcgtgaaccagcacctgtgcggctcccacctggtggaagctctggcactcgtgtgcggcgagcggggcttccactacgggggtggcggaggaggttctggtggcggcggaggcatcgtggaacagtgctgcacctccacctgctccctggaccagctggaaaactactgcggtggcggaggtggtcaaggaggcggtggacagggtggaggtgggcagggaggaggcgggggagacaaaactcacacatgcccaccgtgcccagcacctgaactcctggggggaccgtcagtcttcctcttccccccaaaacccaaggacaccctcatgatctcccggacccctgaggtcacatgcgtggtggtggacgtgagccacgaagaccctgaggtcaagttcaactggtacgtggacggcgtggaggtgcataatgccaagacaaagccgcgggaggagcagtacagaagcacgtaccgtgtggtcagcgtcctcaccgtcctgcaccaggactggctgaatggcaaggagtacaagtgcaaggtctccaacaaagccctcccagcccccatcgagaaaaccatctccaaagccaaagggcagccccgagaaccacaggtgtacaccctgcccccatcccgggatgagctgaccaagaaccaggtcagcctgacctgcctggtcaaaggcttctatcccagcgacatcgccgtggagtgggagagcaatgggcagccggagaacaactacaagaccacgcctcccgtgctggactccgacggctccttcttcctctacagcaagctcaccgtggacaagagcaggtggcagcaggggaacgtcttctcatgctccgtgatgcatgaggctctgcacaaccactacacgcagaagagcctctccctgtctccgggttag

SEQ ID NO: 86 - protein, 304 aa, Artificial Sequence
  Insulin-Fc Fusion Protein
FVNQHLCGSHLVEALALVCGERGFHYGGGGGGSGGGGGIVEQCCTSTCSLDQLENYCGGGGGQGGGGQGGGGQGGGGGDKTHTCPPCPAPELLGGPSVFLFPPKPKDTLMISRTPEVTCVVVDVSHEDPEVKFNWYVDGVEVHNAKTKPREEQYQSTYRVVSVLTVLHQDWLNGKEYKCKVSNKALPAPIEKTISKAKGQPREPQVYTLPPSRDELTKNQVSLTCLVKGFYPSDIAVEWESNGQPENNYKTTPPVLDSDGSFFLYSKLTVDKSRWQQGNVFSCSVMHEALHNHYTQKSLSLSPG

SEQ ID NO: 87 - protein, 304 aa, Artificial Sequence
  Insulin-Fc Fusion Protein
FVNQHLCGSHLVEALALVCGERGFHYGGGGGGSGGGGGIVEQCCTSTCSLDQLENYCGGGGGAGGGGAGGGGAGGGGGDKTHTCPPCPAPELLGGPSVFLFPPKPKDTLMISRTPEVTCVVVDVSHEDPEVKFNWYVDGVEVHNAKTKPREEQYSSTYRVVSVLTVLHQDWLNGKEYKCKVSNKALPAPIEKTISKAKGQPREPQVYTLPPSRDELTKNQVSLTCLVKGFYPSDIAVEWESNGQPENNYKTTPPVLDSDGSFFLYSKLTVDKSRWQQGNVFSCSVMHEALHNHYTQKSLSLSPG

SEQ ID NO: 88 - DNA, 972 bp, Artificial Sequence
  cDNA for Insulin-Fc Fusion Protein
atggaatggagctgggtctttctcttcttcctgtcagtaacgactggtgtccactccttcgtgaaccagcacctgtgcggctcccacctggtggaagctctggcactcgtgtgcggcgagcggggcttccactacgggggtggcggaggaggttctggtggcggcggaggcatcgtggaacagtgctgcacctccacctgctccctggaccagctggaaaactactgcggtggcggaggtggtgcaggaggcggtggagccggtggaggtggggctggaggaggcgggggagacaaaactcacacatgcccaccgtgcccagcacctgaactcctggggggaccgtcagtcttcctcttccccccaaaacccaaggacaccctcatgatctcccggacccctgaggtcacatgcgtggtggtggacgtgagccacgaagaccctgaggtcaagttcaactggtacgtggacggcgtggaggtgcataatgccaagacaaagccgcgggaggagcagtacagcagcacgtaccgtgtggtcagcgtcctcaccgtcctgcaccaggactggctgaatggcaaggagtacaagtgcaaggtctccaacaaagccctcccagcccccatcgagaaaaccatctccaaagccaaagggcagccccgagaaccacaggtgtacaccctgcccccatcccgggatgagctgaccaagaaccaggtcagcctgacctgcctggtcaaaggcttctatcccagcgacatcgccgtggagtgggagagcaatgggcagccggagaacaactacaagaccacgcctcccgtgctggactccgacggctccttcttcctctacagcaagctcaccgtggacaagagcaggtggcagcaggggaacgtcttctcatgctccgtgatgcatgaggctctgcacaaccactacacgcagaagagcctctccctgtctccgggttag

SEQ ID NO: 89 - protein, 292 aa, Artificial Sequence
  Insulin-Fc Fusion Protein
FVNQHLCGSHLVEALALVCGERGFHYGGGGGGSGGGGGIVEQCCTSTCSLDQLENYCGGGGAGGGGDKTHTCPPCPAPELLGGPSVFLFPPKPKDTLMISRTPEVTCVVVDVSHEDPEVKFNWYVDGVEVHNAKTKPREEQYSSTYRVVSVLTVLHQDWLNGKEYKCKVSNKALPAPIEKTISKAKGQPREPQVYTLPPSRDELTKNQVSLTCLVKGFYPSDIAVEWESNGQPENNYKTTPPVLDSDGSFFLYSKLTVDKSRWQQGNVFSCSVMHEALHNHYTQKSLSLSPG

SEQ ID NO: 90 - DNA, 936 bp, Artificial Sequence
  cDNA for Insulin-Fc Fusion Protein
atggaatggagctgggtctttctcttcttcctgtcagtaacgactggtgtccactccttcgtgaaccagcacctgtgcggctcccacctggtggaagctctggcactcgtgtgcggcgagcggggcttccactacgggggtggcggaggaggttctggtggcggcggaggcatcgtggaacagtgctgcacctccacctgctccctggaccagctggaaaactactgcggtggcggaggtgccggaggcgggggagacaaaactcacacatgcccaccgtgcccagcacctgaactcctggggggaccgtcagtcttcctcttccccccaaaacccaaggacaccctcatgatctcccggacccctgaggtcacatgcgtggtggtggacgtgagccacgaagaccctgaggtcaagttcaactggtacgtggacggcgtggaggtgcataatgccaagacaaagccgcgggaggagcagtacagcagcacgtaccgtgtggtcagcgtcctcaccgtcctgcaccaggactggctgaatggcaaggagtacaagtgcaaggtctccaacaaagccctcccagcccccatcgagaaaaccatctccaaagccaaagggcagccccgagaaccacaggtgtacaccctgcccccatcccgggatgagctgaccaagaaccaggtcagcctgacctgcctggtcaaaggcttctatcccagcgacatcgccgtggagtgggagagcaatgggcagccggagaacaactacaagaccacgcctcccgtgctggactccgacggctccttcttcctctacagcaagctcaccgtggacaagagcaggtggcagcaggggaacgtcttctcatgctccgtgatgcatgaggctctgcacaaccactacacgcagaagagcctctccctgtctccgggttag

SEQ ID NO: 91 - protein, 304 aa, Artificial Sequence
  Insulin-Fc Fusion Protein
FVNQHLCGSHLVEALELVCGERGFHYGGGGGGSGGGGGIVEQCCTSTCSLDQLENYCGGGGGQGGGGQGGGGQGGGGGDKTHTCPPCPAPELLGGPSVFLFPPKPKDTLMISRTPEVTCVVVDVSHEDPEVKFNWYVDGVEVHNAKTKPREEQYSSTYRVVSVLTVLHQDWLNGKEYKCKVSNKALPAPIEKTISKAKGQPREPQVYTLPPSRDELTKNQVSLTCLVKGFYPSDIAVEWESNGQPENNYKTTPPVLDSDGSFFLYSKLTVDKSRWQQGNVFSCSVMHEALHNHYTQKSLSLSPG

SEQ ID NO: 92 - protein, 304 aa, Artificial Sequence
  Insulin-Fc Fusion Protein
FVNQHLCGSHLVEALELVCGERGFHYGGGGGGSGGGGGIVEQCCTSTCSLDQLENYCGGGGGQGGGGQGGGGQGGGGGDKTHTCPPCPAPELLGGPSVFLFPPKPKDTLMISRTPEVTCVVVDVSHEDPEVKFNWYVDGVEVHNAKTKPREEQYDSTYRVVSVLTVLHQDWLNGKEYKCKVSNKALPAPIEKTISKAKGQPREPQVYTLPPSRDELTKNQVSLTCLVKGFYPSDIAVEWESNGQPENNYKTTPPVLDSDGSFFLYSKLTVDKSRWQQGNVFSCSVMHEALHNHYTQKSLSLSPG

SEQ ID NO: 93 - protein, 304 aa, Artificial Sequence
  Insulin-Fc Fusion Protein
FVNQHLCGSHLVEALELVCGERGFHYGGGGGGSGGGGGIVEQCCTSTCSLDQLENYCGGGGGQGGGGQGGGGQGGGGGDKTHTCPPCPAPELLGGPSVFLFPPKPKDTLMISRTPEVTCVVVDVSHEDPEVKFNWYVDGVEVHNAKTKPREEQYASTYRVVSVLTVLHQDWLNGKEYKCKVSNKALPAPIEKTISKAKGQPREPQVYTLPPSRDELTKNQVSLTCLVKGFYPSDIAVEWESNGQPENNYKTTPPVLDSDGSFFLYSKLTVDKSRWQQGNVFSCSVMHEALHNHYTQKSLSLSPG

SEQ ID NO: 94 - protein, 304 aa, Artificial Sequence
  Insulin-Fc Fusion Protein
FVNQHLCGSHLVEALELVCGERGFHYGGGGGGSGGGGGIVEQCCTSTCSLDQLENYCGGGGGQGGGGQGGGGQGGGGGDKTHTCPPCPAPELLGGPSVFLFPPKPKDTLMISRTPEVTCVVVDVSHEDPEVKFNWYVDGVEVHNAKTKPREEQYRSTYRVVSVLTVLHQDWLNGKEYKCKVSNKALPAPIEKTISKAKGQPREPQVYTLPPSRDELTKNQVSLTCLVKGFYPSDIAVEWESNGQPENNYKTTPPVLDSDGSFFLYSKLTVDKSRWQQGNVFSCSVMHEALHNHYTQKSLSLSPG

SEQ ID NO: 95 - protein, 304 aa, Artificial Sequence
  Insulin-Fc Fusion Protein
FVNQHLCGSHLVEALELVCGERGFHYGGGGGGSGGGGGIVEQCCTSTCSLDQLENYCGGGGGQGGGGQGGGGQGGGGGDKTHTCPPCPAPELLGGPSVFLFPPKPKDTLMISRTPEVTCVVVDVSHEDPEVKFNWYVDGVEVHNAKTKPREEQYQSTYRVVSVLTVLHQDWLNGKEYKCKVSNKALPAPIEKTISKAKGQPREPQVYTLPPSRDELTKNQVSLTCLVKGFYPSDIAVEWESNGQPENNYKTTPPVLDSDGSFFLYSKLTVDKSRWQQGNVFSCSVMHEALHNHYTQKSLSLSPG

SEQ ID NO: 96 - protein, 309 aa, Artificial Sequence
  Insulin-Fc Fusion Protein
FVNQHLCGSHLVEALALVCGERGFHYGGGGGGSGGGGGIVEQCCTSTCSLDQLENYCGGGGGQGGGGQGGGGQGGGGGQGGGGDKTHTCPPCPAPELLGGPSVFLFPPKPKDTLMISRTPEVTCVVVDVSHEDPEVKFNWYVDGVEVHNAKTKPREEQYSSTYRVVSVLTVLHQDWLNGKEYKCKVSNKALPAPIEKTISKAKGQPREPQVYTLPPSRDELTKNQVSLTCLVKGFYPSDIAVEWESNGQPENNYKTTPPVLDSDGSFFLYSKLTVDKSRWQQGNVFSCSVMHEALHNHYTQKSLSLSPG

SEQ ID NO: 97 - protein, 292 aa, Artificial Sequence
  Insulin-Fc Fusion Protein
FVNQHLCGSHLVEALALVCGERGFHYGGGGGGSGGGGGIVEQCCTSTCSLDQLENYCGGGGQGGGGDKTHTCPPCPAPELLGGPSVFLFPPKPKDTLMISRTPEVTCVVVDVSHEDPEVKFNWYVDGVEVHNAKTKPREEQYSSTYRVVSVLTVLHQDWLNGKEYKCKVSNKALPAPIEKTISKAKGQPREPQVYTLPPSRDELTKNQVSLTCLVKGFYPSDIAVEWESNGQPENNYKTTPPVLDSDGSFFLYSKLTVDKSRWQQGNVFSCSVMHEALHNHYTQKSLSLSPG

SEQ ID NO: 98 - protein, 283 aa, Artificial Sequence
  Insulin-Fc Fusion Protein
FVNQHLCGSHLVEALALVCGERGFHYGGGGGGSGGGGGIVEQCCTSTCSLDQLENYCDKTHTCPPCPAPELLGGPSVFLFPPKPKDTLMISRTPEVTCVVVDVSHEDPEVKFNWYVDGVEVHNAKTKPREEQYSSTYRVVSVLTVLHQDWLNGKEYKCKVSNKALPAPIEKTISKAKGQPREPQVYTLPPSRDELTKNQVSLTCLVKGFYPSDIAVEWESNGQPENNYKTTPPVLDSDGSFFLYSKLTVDKSRWQQGNVFSCSVMHEALHNHYTQKSLSLSPG

SEQ ID NO: 99 - protein, 26 aa, Artificial Sequence
  Linker
GGGGGQGGGGQGGGGQGGGGGQGGGG

SEQ ID NO: 100 - DNA, 972 bp, Artificial Sequence
  cDNA for Insulin-Fc Fusion Protein
atggaatggagctgggtctttctcttcttcctgtcagtaacgactggtgtccactccttcgtgaaccagcacctgtgcggctcccacctggtggaagctctggcactcgtgtgcggcgagcggggcttccactacgggggtggcggaggaggttctggtggcggcggaggcatcgtggaacagtgctgcacctccacctgctccctggaccagctggaaaactactgcggtggcggaggtggtcaaggaggcggtggacagggtggaggtgggcagggaggaggcgggggagacaaaactcacacatgcccaccgtgcccagcacctgaactcctggggggaccgtcagtcttcctcttccccccaaaacccaaggacaccctcatgatctcccggacccctgaggtcacatgcgtggtggtggacgtgagccacgaagaccctgaggtcaagttcaactggtacgtggacggcgtggaggtgcataatgccaagacaaagccgcgggaggagcagtaccaaagcacgtaccgtgtggtcagcgtcctcaccgtcctgcaccaggactggctgaatggcaaggagtacaagtgcaaggtctccaacaaagccctcccagcccccatcgagaaaaccatctccaaagccaaagggcagccccgagaaccacaggtgtacaccctgcccccatcccgggatgagctgaccaagaaccaggtcagcctgacctgcctggtcaaaggcttctatcccagcgacatcgccgtggagtgggagagcaatgggcagccggagaacaactacaagaccacgcctcccgtgctggactccgacggctccttcttcctctacagcaagctcaccgtggacaagagcaggtggcagcaggggaacgtcttctcatgctccgtgatgcatgaggctctgcacaaccactacacgcagaagagcctctccctgtctccgggttag